European Patent Application EP 4 180 453 A1, published May 17, 2023. Title: FUSION PROTEIN COMPRISING COMPLEMENT PATHWAY INHIBITOR AND ANGIOGENESIS INHIBITOR AND USE THEREOF. Applicant: Kanaph Therapeutics. The sequence listing filed with the application follows.

SEQUENCE LISTING (151 sequences)

SEQ ID NO: 1 - protein, 496 aa, Artificial Sequence
  hu CRIg-hu IgG1 Fc DANG
RPILEVPESVTGPWKGDVNLPCTYDPLQGYTQVLVKWLVQRGSDPVTIFLRDSSGDHIQQAKYQGRLHVSHKVPGDVSLQLSTLEMDDRSHYTCEVTWQTPDGNQVVRDKITELRVQKLSVSKPTVTTGSGYGFTVPQGMRISLQCQARGSPPISYIWYKQQTNNQEPIKVATLSTLLFKPAVIADSGSYFCTAKGQVGSEQHSDIVKFVVKDSSKLLKTKTEAPTTMTYPLKATSTVKQSWDWTTDMDGYLGETSAGPGKSLPGGGGSDKTHTCPPCPAPELLGGPSVFLFPPKPKDTLMISRTPEVTCVVVAVSHEDPEVKFNWYVDGVEVHNAKTKPREEQYGSTYRVVSVLTVLHQDWLNGKEYKCKVSNKALPAPIEKTISKAKGQPREPQVYTLPPSRDELTKNQVSLTCLVKGFYPSDIAVEWESNGQPENNYKTTPPVLDSDGSFFLYSKLTVDKSRWQQGNVFSCSVMHEALHNHYTQKSLSLSPGK

SEQ ID NO: 2 - protein, 710 aa, Artificial Sequence
  hu CRIg-hu IgG1 Fc DANG-VEGF binder
RPILEVPESVTGPWKGDVNLPCTYDPLQGYTQVLVKWLVQRGSDPVTIFLRDSSGDHIQQAKYQGRLHVSHKVPGDVSLQLSTLEMDDRSHYTCEVTWQTPDGNQVVRDKITELRVQKLSVSKPTVTTGSGYGFTVPQGMRISLQCQARGSPPISYIWYKQQTNNQEPIKVATLSTLLFKPAVIADSGSYFCTAKGQVGSEQHSDIVKFVVKDSSKLLKTKTEAPTTMTYPLKATSTVKQSWDWTTDMDGYLGETSAGPGKSLPGGGGSDKTHTCPPCPAPELLGGPSVFLFPPKPKDTLMISRTPEVTCVVVAVSHEDPEVKFNWYVDGVEVHNAKTKPREEQYGSTYRVVSVLTVLHQDWLNGKEYKCKVSNKALPAPIEKTISKAKGQPREPQVYTLPPSRDELTKNQVSLTCLVKGFYPSDIAVEWESNGQPENNYKTTPPVLDSDGSFFLYSKLTVDKSRWQQGNVFSCSVMHEALHNHYTQKSLSLSPGGGGGSGGGGSSDTGRPFVEMYSEIPEIIHMTEGRELVIPCRVTSPNITVTLKKFPLDTLIPDGKRIIWDSRKGFIISNATYKEIGLLTCEATVNGHLYKTNYLTHRQTNTIIDVVLSPSHGIELSVGEKLVLNCTARTELNVGIDFNWEYPSSKHQHKKLVNRDLKTQSGSEMKKFLSTLTIDGVTRSDQGLYTCAASSGLMTKKNSTFVRVHEK

SEQ ID NO: 3 - protein, 501 aa, Artificial Sequence
  hu IgG1 Fc DANG-hu CRIg
DKTHTCPPCPAPELLGGPSVFLFPPKPKDTLMISRTPEVTCVVVAVSHEDPEVKFNWYVDGVEVHNAKTKPREEQYGSTYRVVSVLTVLHQDWLNGKEYKCKVSNKALPAPIEKTISKAKGQPREPQVYTLPPSRDELTKNQVSLTCLVKGFYPSDIAVEWESNGQPENNYKTTPPVLDSDGSFFLYSKLTVDKSRWQQGNVFSCSVMHEALHNHYTQKSLSLSPGGGGGSGGGGSRPILEVPESVTGPWKGDVNLPCTYDPLQGYTQVLVKWLVQRGSDPVTIFLRDSSGDHIQQAKYQGRLHVSHKVPGDVSLQLSTLEMDDRSHYTCEVTWQTPDGNQVVRDKITELRVQKLSVSKPTVTTGSGYGFTVPQGMRISLQCQARGSPPISYIWYKQQTNNQEPIKVATLSTLLFKPAVIADSGSYFCTAKGQVGSEQHSDIVKFVVKDSSKLLKTKTEAPTTMTYPLKATSTVKQSWDWTTDMDGYLGETSAGPGKSLPG

SEQ ID NO: 4 - protein, 711 aa, Artificial Sequence
  VEGF binder-hu IgG1 Fc DANG-hu CRIg
SDTGRPFVEMYSEIPEIIHMTEGRELVIPCRVTSPNITVTLKKFPLDTLIPDGKRIIWDSRKGFIISNATYKEIGLLTCEATVNGHLYKTNYLTHRQTNTIIDVVLSPSHGIELSVGEKLVLNCTARTELNVGIDFNWEYPSSKHQHKKLVNRDLKTQSGSEMKKFLSTLTIDGVTRSDQGLYTCAASSGLMTKKNSTFVRVHEKGGGGSDKTHTCPPCPAPELLGGPSVFLFPPKPKDTLMISRTPEVTCVVVAVSHEDPEVKFNWYVDGVEVHNAKTKPREEQYGSTYRVVSVLTVLHQDWLNGKEYKCKVSNKALPAPIEKTISKAKGQPREPQVYTLPPSRDELTKNQVSLTCLVKGFYPSDIAVEWESNGQPENNYKTTPPVLDSDGSFFLYSKLTVDKSRWQQGNVFSCSVMHEALHNHYTQKSLSLSPGGGGGSGGGGSRPILEVPESVTGPWKGDVNLPCTYDPLQGYTQVLVKWLVQRGSDPVTIFLRDSSGDHIQQAKYQGRLHVSHKVPGDVSLQLSTLEMDDRSHYTCEVTWQTPDGNQVVRDKITELRVQKLSVSKPTVTTGSGYGFTVPQGMRISLQCQARGSPPISYIWYKQQTNNQEPIKVATLSTLLFKPAVIADSGSYFCTAKGQVGSEQHSDIVKFVVKDSSKLLKTKTEAPTTMTYPLKATSTVKQSWDWTTDMDGYLGETSAGPGKSLPG

SEQ ID NO: 5 - protein, 436 aa, Artificial Sequence
  VEGF binder-hu IgG1 Fc DANG
SDTGRPFVEMYSEIPEIIHMTEGRELVIPCRVTSPNITVTLKKFPLDTLIPDGKRIIWDSRKGFIISNATYKEIGLLTCEATVNGHLYKTNYLTHRQTNTIIDVVLSPSHGIELSVGEKLVLNCTARTELNVGIDFNWEYPSSKHQHKKLVNRDLKTQSGSEMKKFLSTLTIDGVTRSDQGLYTCAASSGLMTKKNSTFVRVHEKGGGGSDKTHTCPPCPAPELLGGPSVFLFPPKPKDTLMISRTPEVTCVVVAVSHEDPEVKFNWYVDGVEVHNAKTKPREEQYGSTYRVVSVLTVLHQDWLNGKEYKCKVSNKALPAPIEKTISKAKGQPREPQVYTLPPSRDELTKNQVSLTCLVKGFYPSDIAVEWESNGQPENNYKTTPPVLDSDGSFFLYSKLTVDKSRWQQGNVFSCSVMHEALHNHYTQKSLSLSPG

SEQ ID NO: 6 - protein, 208 aa, Artificial Sequence
  hu IgG1 Fc DANG
SVFLFPPKPKDTLMISRTPEVTCVVVAVSHEDPEVKFNWYVDGVEVHNAKTKPREEQYGSTYRVVSVLTVLHQDWLNGKEYKCKVSNKALPAPIEKTISKAKGQPREPQVYTLPPSRDELTKNQVSLTCLVKGFYPSDIAVEWESNGQPENNYKTTPPVLDSDGSFFLYSKLTVDKSRWQQGNVFSCSVMHEALHNHYTQKSLSLSPG

SEQ ID NO: 7 - protein, 406 aa, Artificial Sequence
  mu CRIg-mu IgG2a Fc DANG
HPTLKTPESVTGTWKGDVKIQCIYDPLRGYRQVLVKWLVRHGSDSVTIFLRDSTGDHIQQAKYRGRLKVSHKVPGDVSLQINTLQMDDRNHYTCEVTWQTPDGNQVIRDKIIELRVRKYNPPRINTEAPTTLHSSLEATTIMSSTSDLTTNGTGKLEETIAGSGRNLPGGGGSEPRGPTIKPCPPCKCPAPNLLGGPSVFIFPPKIKDVLMISLSPIVTCVVVAVSEDDPDVQISWFVNNVEVHTAQTQTHREDYGSTLRVVSALPIQHQDWMSGKEFKCKVNNKDLPAPIERTISKPKGSVRAPQVYVLPPPEEEMTKKQVTLTCMVTDFMPEDIYVEWTNNGKTELNYKNTEPVLDSDGSYFMYSKLRVEKKNWVERNSYSCSVVHEGLHNHHTTKSFSRTPGK

SEQ ID NO: 8 - protein, 620 aa, Artificial Sequence
  mu CRIg-mu IgG2a Fc DANG-VEGF binder
HPTLKTPESVTGTWKGDVKIQCIYDPLRGYRQVLVKWLVRHGSDSVTIFLRDSTGDHIQQAKYRGRLKVSHKVPGDVSLQINTLQMDDRNHYTCEVTWQTPDGNQVIRDKIIELRVRKYNPPRINTEAPTTLHSSLEATTIMSSTSDLTTNGTGKLEETIAGSGRNLPGGGGSEPRGPTIKPCPPCKCPAPNLLGGPSVFIFPPKIKDVLMISLSPIVTCVVVAVSEDDPDVQISWFVNNVEVHTAQTQTHREDYGSTLRVVSALPIQHQDWMSGKEFKCKVNNKDLPAPIERTISKPKGSVRAPQVYVLPPPEEEMTKKQVTLTCMVTDFMPEDIYVEWTNNGKTELNYKNTEPVLDSDGSYFMYSKLRVEKKNWVERNSYSCSVVHEGLHNHHTTKSFSRTPGGGGGSGGGGSSDTGRPFVEMYSEIPEIIHMTEGRELVIPCRVTSPNITVTLKKFPLDTLIPDGKRIIWDSRKGFIISNATYKEIGLLTCEATVNGHLYKTNYLTHRQTNTIIDVVLSPSHGIELSVGEKLVLNCTARTELNVGIDFNWEYPSSKHQHKKLVNRDLKTQSGSEMKKFLSTLTIDGVTRSDQGLYTCAASSGLMTKKNSTFVRVHEK

SEQ ID NO: 9 - protein, 411 aa, Artificial Sequence
  mu IgG2a Fc DANG-mu CRIg
EPRGPTIKPCPPCKCPAPNLLGGPSVFIFPPKIKDVLMISLSPIVTCVVVAVSEDDPDVQISWFVNNVEVHTAQTQTHREDYGSTLRVVSALPIQHQDWMSGKEFKCKVNNKDLPAPIERTISKPKGSVRAPQVYVLPPPEEEMTKKQVTLTCMVTDFMPEDIYVEWTNNGKTELNYKNTEPVLDSDGSYFMYSKLRVEKKNWVERNSYSCSVVHEGLHNHHTTKSFSRTPGGGGGSGGGGSHPTLKTPESVTGTWKGDVKIQCIYDPLRGYRQVLVKWLVRHGSDSVTIFLRDSTGDHIQQAKYRGRLKVSHKVPGDVSLQINTLQMDDRNHYTCEVTWQTPDGNQVIRDKIIELRVRKYNPPRINTEAPTTLHSSLEATTIMSSTSDLTTNGTGKLEETIAGSGRNLPG

SEQ ID NO: 10 - protein, 621 aa, Artificial Sequence
  VEGF binder-mu IgG2a Fc DANG-mu CRIg
SDTGRPFVEMYSEIPEIIHMTEGRELVIPCRVTSPNITVTLKKFPLDTLIPDGKRIIWDSRKGFIISNATYKEIGLLTCEATVNGHLYKTNYLTHRQTNTIIDVVLSPSHGIELSVGEKLVLNCTARTELNVGIDFNWEYPSSKHQHKKLVNRDLKTQSGSEMKKFLSTLTIDGVTRSDQGLYTCAASSGLMTKKNSTFVRVHEKGGGGSEPRGPTIKPCPPCKCPAPNLLGGPSVFIFPPKIKDVLMISLSPIVTCVVVAVSEDDPDVQISWFVNNVEVHTAQTQTHREDYGSTLRVVSALPIQHQDWMSGKEFKCKVNNKDLPAPIERTISKPKGSVRAPQVYVLPPPEEEMTKKQVTLTCMVTDFMPEDIYVEWTNNGKTELNYKNTEPVLDSDGSYFMYSKLRVEKKNWVERNSYSCSVVHEGLHNHHTTKSFSRTPGGGGGSGGGGSHPTLKTPESVTGTWKGDVKIQCIYDPLRGYRQVLVKWLVRHGSDSVTIFLRDSTGDHIQQAKYRGRLKVSHKVPGDVSLQINTLQMDDRNHYTCEVTWQTPDGNQVIRDKIIELRVRKYNPPRINTEAPTTLHSSLEATTIMSSTSDLTTNGTGKLEETIAGSGRNLPG

SEQ ID NO: 11 - protein, 217 aa, Artificial Sequence
  mu IgG2a Fc DANG
APNLLGGPSVFIFPPKIKDVLMISLSPIVTCVVVAVSEDDPDVQISWFVNNVEVHTAQTQTHREDYGSTLRVVSALPIQHQDWMSGKEFKCKVNNKDLPAPIERTISKPKGSVRAPQVYVLPPPEEEMTKKQVTLTCMVTDFMPEDIYVEWTNNGKTELNYKNTEPVLDSDGSYFMYSKLRVEKKNWVERNSYSCSVVHEGLHNHHTTKSFSRTPGK

SEQ ID NO: 12 - protein, 447 aa, Artificial Sequence
  mu IgG2a Fc DANG-VEGF binder
EPRGPTIKPCPPCKCPAPNLLGGPSVFIFPPKIKDVLMISLSPIVTCVVVAVSEDDPDVQISWFVNNVEVHTAQTQTHREDYGSTLRVVSALPIQHQDWMSGKEFKCKVNNKDLPAPIERTISKPKGSVRAPQVYVLPPPEEEMTKKQVTLTCMVTDFMPEDIYVEWTNNGKTELNYKNTEPVLDSDGSYFMYSKLRVEKKNWVERNSYSCSVVHEGLHNHHTTKSFSRTPGGGGGSGGGGSSDTGRPFVEMYSEIPEIIHMTEGRELVIPCRVTSPNITVTLKKFPLDTLIPDGKRIIWDSRKGFIISNATYKEIGLLTCEATVNGHLYKTNYLTHRQTNTIIDVVLSPSHGIELSVGEKLVLNCTARTELNVGIDFNWEYPSSKHQHKKLVNRDLKTQSGSEMKKFLSTLTIDGVTRSDQGLYTCAASSGLMTKKNSTFVRVHEK

SEQ ID NO: 13 - protein, 431 aa, Artificial Sequence
  Aflibercept
SDTGRPFVEMYSEIPEIIHMTEGRELVIPCRVTSPNITVTLKKFPLDTLIPDGKRIIWDSRKGFIISNATYKEIGLLTCEATVNGHLYKTNYLTHRQTNTIIDVVLSPSHGIELSVGEKLVLNCTARTELNVGIDFNWEYPSSKHQHKKLVNRDLKTQSGSEMKKFLSTLTIDGVTRSDQGLYTCAASSGLMTKKNSTFVRVHEKDKTHTCPPCPAPELLGGPSVFLFPPKPKDTLMISRTPEVTCVVVDVSHEDPEVKFNWYVDGVEVHNAKTKPREEQYNSTYRVVSVLTVLHQDWLNGKEYKCKVSNKALPAPIEKTISKAKGQPREPQVYTLPPSRDELTKNQVSLTCLVKGFYPSDIAVEWESNGQPENNYKTTPPVLDSDGSFFLYSKLTVDKSRWQQGNVFSCSVMHEALHNHYTQKSLSLSPG

SEQ ID NO: 14 - protein, 205 aa, Artificial Sequence
  VEGF binder (VEGFR1 D2-VEGFR2 D3)
SDTGRPFVEMYSEIPEIIHMTEGRELVIPCRVTSPNITVTLKKFPLDTLIPDGKRIIWDSRKGFIISNATYKEIGLLTCEATVNGHLYKTNYLTHRQTNTIIDVVLSPSHGIELSVGEKLVLNCTARTELNVGIDFNWEYPSSKHQHKKLVNRDLKTQSGSEMKKFLSTLTIDGVTRSDQGLYTCAASSGLMTKKNSTFVRVHEK

SEQ ID NO: 15 - protein, 23 aa, Artificial Sequence
  human linker-1
GGGGSDKTHTCPPCPAPELLGGP

SEQ ID NO: 16 - protein, 10 aa, Artificial Sequence
  linker-2
GGGGSGGGGS

SEQ ID NO: 17 - protein, 21 aa, Artificial Sequence
  mouse linker-1
GGGGSEPRGPTIKPCPPCKCP

SEQ ID NO: 18 - protein, 5 aa, Artificial Sequence
  linker-2
GGGGS

SEQ ID NO: 19 - protein, 399 aa, Artificial Sequence
  Human CRIg-Whole
MGILLGLLLLGHLTVDTYGRPILEVPESVTGPWKGDVNLPCTYDPLQGYTQVLVKWLVQRGSDPVTIFLRDSSGDHIQQAKYQGRLHVSHKVPGDVSLQLSTLEMDDRSHYTCEVTWQTPDGNQVVRDKITELRVQKLSVSKPTVTTGSGYGFTVPQGMRISLQCQARGSPPISYIWYKQQTNNQEPIKVATLSTLLFKPAVIADSGSYFCTAKGQVGSEQHSDIVKFVVKDSSKLLKTKTEAPTTMTYPLKATSTVKQSWDWTTDMDGYLGETSAGPGKSLPVFAIILIISLCCMVVFTMAYIMLCRKTSQQEHVYEAARAHAREANDSGETMRVAIFASGCSSDEPTSQNLGNNYSDEPCIGQEYQIIAQINGNYARLLDTVPLDYEFLATEGKSVC

SEQ ID NO: 20 - protein, 305 aa, Artificial Sequence
  human CRIg(VSIG4) isoform 3
MGILLGLLLLGHLTVDTYGRPILEVPESVTGPWKGDVNLPCTYDPLQGYTQVLVKWLVQRGSDPVTIFLRDSSGDHIQQAKYQGRLHVSHKVPGDVSLQLSTLEMDDRSHYTCEVTWQTPDGNQVVRDKITELRVQKHSSKLLKTKTEAPTTMTYPLKATSTVKQSWDWTTDMDGYLGETSAGPGKSLPVFAIILIISLCCMVVFTMAYIMLCRKTSQQEHVYEAARAHAREANDSGETMRVAIFASGCSSDEPTSQNLGNNYSDEPCIGQEYQIIAQINGNYARLLDTVPLDYEFLATEGKSVC

SEQ ID NO: 21 - protein, 280 aa, Artificial Sequence
  mouse CRIg whole
MEISSGLLFLGHLIVLTYGHPTLKTPESVTGTWKGDVKIQCIYDPLRGYRQVLVKWLVRHGSDSVTIFLRDSTGDHIQQAKYRGRLKVSHKVPGDVSLQINTLQMDDRNHYTCEVTWQTPDGNQVIRDKIIELRVRKYNPPRINTEAPTTLHSSLEATTIMSSTSDLTTNGTGKLEETIAGSGRNLPIFAIIFIISLCCIVAVTIPYILFRCRTFQQEYVYGVSRVFARKTSNSEETTRVTTIATDEPDSQALISDYSDDPCLSQEYQITIRSTMSIPAC

SEQ ID NO: 22 - protein, 264 aa, Artificial Sequence
  Extracellular Domain of human CRIg
RPILEVPESVTGPWKGDVNLPCTYDPLQGYTQVLVKWLVQRGSDPVTIFLRDSSGDHIQQAKYQGRLHVSHKVPGDVSLQLSTLEMDDRSHYTCEVTWQTPDGNQVVRDKITELRVQKLSVSKPTVTTGSGYGFTVPQGMRISLQCQARGSPPISYIWYKQQTNNQEPIKVATLSTLLFKPAVIADSGSYFCTAKGQVGSEQHSDIVKFVVKDSSKLLKTKTEAPTTMTYPLKATSTVKQSWDWTTDMDGYLGETSAGPGKSLP

SEQ ID NO: 23 - DNA, 1488 bp, Artificial Sequence
  nucleotide sequence of hu CRIg-hu IgG1 Fc DANG
cggcctatcctggaggtgccagagtccgtgaccggaccatggaagggcgacgtgaacctgccctgcacctacgatcctctgcagggctatacacaggtgctggtgaagtggctggtgcagaggggcagcgaccctgtgaccatcttcctgcgcgacagctccggcgatcacatccagcaggccaagtaccagggcaggctgcacgtgtctcacaaggtgcctggcgatgtgagcctgcagctgtccaccctggagatggacgatcgcagccactatacatgtgaggtgacctggcagacaccagacggcaatcaggtggtgcgggataagatcaccgagctgagagtgcagaagctgtccgtgtctaagccaaccgtgaccacaggcagcggctacggcttcacagtgccccagggcatgaggatctccctgcagtgccaggcaaggggctctccacctatcagctacatctggtataagcagcagaccaacaatcaggagcctatcaaggtggccaccctgtccacactgctgttcaagccagccgtgatcgccgacagcggctcctatttttgtacagcaaagggacaagtgggctccgagcagcactctgacatcgtgaagtttgtggtgaaggattctagcaagctgctgaagaccaagacagaggcccctaccacaatgacctacccactgaaggccaccagcacagtgaagcagtcctgggactggaccacagacatggatggctatctgggcgagacatctgccggaccaggcaagagcctgccaggaggaggcggcagcgataagacccacacatgcccaccctgtcctgcaccagagctgctgggaggaccatccgtgttcctgtttcctccaaagcctaaggacaccctgatgatctctcggaccccagaggtgacatgcgtggtggtggccgtgagccacgaggaccccgaggtgaagtttaactggtacgtggatggcgtggaggtgcacaatgccaagaccaagccccgggaggagcagtacggctccacctatagagtggtgtctgtgctgacagtgctgcaccaggattggctgaacggcaaggagtataagtgcaaggtgtccaataaggccctgcccgcccctatcgagaagaccatctctaaggcaaagggacagccaagggagccacaggtgtacacactgcccccttccagagacgagctgaccaagaaccaggtgtctctgacatgtctggtgaagggcttctatccctctgatatcgccgtggagtgggagagcaatggccagcctgagaacaattacaagaccacaccacccgtgctggactccgatggctctttctttctgtatagcaagctgaccgtggataagtccagatggcagcagggcaacgtgttttcttgtagcgtgatgcacgaggccctgcacaatcactacacacagaagtccctgtctctgagccccggcaag

SEQ ID NO: 24 - DNA, 2130 bp, Artificial Sequence
  nucleotide sequence of hu CRIg-hu IgG1 Fc DANG-VEGF binder
cgccctatcctggaggtgccagagtccgtgaccggaccatggaagggcgacgtgaacctgccctgcacctacgatcctctgcagggctatacacaggtgctggtgaagtggctggtgcagaggggcagcgaccctgtgaccatcttcctgcgcgacagctccggcgatcacatccagcaggccaagtaccagggcaggctgcacgtgtcccacaaggtgcctggcgacgtgagcctgcagctgtctaccctggagatggacgatcgcagccactatacatgtgaggtgacctggcagacaccagacggcaatcaggtggtgagggataagatcaccgagctgcgcgtgcagaagctgtccgtgtctaagccaaccgtgaccacaggctctggctacggcttcacagtgccccagggcatgaggatcagcctgcagtgccaggcaaggggcagcccacctatctcctacatctggtataagcagcagaccaacaatcaggagcctatcaaggtggccaccctgtccacactgctgttcaagccagccgtgatcgccgacagcggctcctacttttgtacagccaagggccaagtgggctctgagcagcacagcgacatcgtgaagtttgtggtgaaggattctagcaagctgctgaagaccaagacagaggcccctaccacaatgacctacccactgaaggccacctccacagtgaagcagtcttgggactggaccacagacatggatggctatctgggagagacaagcgccggacctggcaagtccctgccaggaggcggcggctccgataagacccacacatgcccaccatgtcctgcaccagagctgctgggaggacctagcgtgttcctgtttcctccaaagccaaaggacaccctgatgatctcccggaccccagaggtgacatgcgtggtggtggccgtgtctcacgaggaccccgaggtgaagttcaactggtacgtggatggcgtggaggtgcacaatgccaagaccaagccccgggaggagcagtacggctctacctatagagtggtgagcgtgctgacagtgctgcaccaggattggctgaacggcaaggagtataagtgcaaggtgagcaataaggccctgcccgcccctatcgagaagaccatctccaaggcaaagggacagccaagggagccacaggtgtacacactgcccccttccagagacgagctgaccaagaaccaggtgtctctgacatgtctggtgaagggcttttatccctctgatatcgccgtggagtgggagagcaatggccagcctgagaacaattacaagaccacaccacccgtgctggactctgatggcagcttctttctgtattccaagctgaccgtggacaagtctagatggcagcagggcaacgtgttctcttgcagcgtgatgcacgaggccctgcacaatcactacacccagaagtccctgtctctgagcccaggaggaggaggaggctctggaggaggaggctcctctgatacaggcaggccctttgtggagatgtatagcgagatccctgagatcatccacatgaccgagggaagggagctggtcatcccatgtagagtgacatcccctaacatcaccgtgacactgaagaagttcccactggacaccctgatccccgatggcaagcggatcatctgggacagcagaaagggctttatcatctccaatgccacatacaaggagatcggcctgctgacctgcgaggccacagtgaacggccacctgtacaagaccaattatctgacacaccgccagaccaacacaatcatcgatgtggtgctgtccccatctcacggcatcgagctgagcgtgggcgagaagctggtgctgaattgtaccgcccggacagagctgaacgtgggcatcgacttcaattgggagtaccctagctccaagcaccagcacaagaagctggtcaaccgggatctgaagacccagagcggctccgagatgaagaagtttctgagcaccctgacaatcgacggcgtgaccagatccgatcagggcctgtatacatgtgccgcctctagcggcctgatgaccaagaagaatagcacatttgtgagggtgcacgagaag

SEQ ID NO: 25 - DNA, 1503 bp, Artificial Sequence
  nucleotide sequence of hu IgG1 Fc DANG-hu CRIg
gataagacccacacatgcccaccctgtcctgcaccagagctgctgggaggaccatccgtgttcctgtttcctccaaagcctaaggacaccctgatgatctctcggaccccagaggtgacatgcgtggtggtggccgtgagccacgaggaccccgaggtgaagtttaactggtacgtggatggcgtggaggtgcacaatgccaagaccaagccccgggaggagcagtacggctccacctatagagtggtgtctgtgctgacagtgctgcaccaggattggctgaacggcaaggagtataagtgcaaggtgtccaataaggccctgcccgcccctatcgagaagaccatctctaaggcaaagggacagccaagggagccacaggtgtacacactgcccccttccagagacgagctgaccaagaaccaggtgtctctgacatgtctggtgaagggcttctatccctctgatatcgccgtggagtgggagagcaatggccagcctgagaacaattacaagaccacaccacccgtgctggactccgatggctctttctttctgtatagcaagctgaccgtggataagtccagatggcagcagggcaacgtgttttcttgtagcgtgatgcacgaggccctgcacaatcactacacacagaagtccctgtctctgagccccggcggcggaggcgggtctggaggtggagggagtcggcctatcctggaggtgccagagtccgtgaccggaccatggaagggcgacgtgaacctgccctgcacctacgatcctctgcagggctatacacaggtgctggtgaagtggctggtgcagaggggcagcgaccctgtgaccatcttcctgcgcgacagctccggcgatcacatccagcaggccaagtaccagggcaggctgcacgtgtctcacaaggtgcctggcgatgtgagcctgcagctgtccaccctggagatggacgatcgcagccactatacatgtgaggtgacctggcagacaccagacggcaatcaggtggtgcgggataagatcaccgagctgagagtgcagaagctgtccgtgtctaagccaaccgtgaccacaggcagcggctacggcttcacagtgccccagggcatgaggatctccctgcagtgccaggcaaggggctctccacctatcagctacatctggtataagcagcagaccaacaatcaggagcctatcaaggtggccaccctgtccacactgctgttcaagccagccgtgatcgccgacagcggctcctatttttgtacagcaaagggacaagtgggctccgagcagcactctgacatcgtgaagtttgtggtgaaggattctagcaagctgctgaagaccaagacagaggcccctaccacaatgacctacccactgaaggccaccagcacagtgaagcagtcctgggactggaccacagacatggatggctatctgggcgagacatctgccggaccaggcaagagcctgccagga

SEQ ID NO: 26 - DNA, 2133 bp, Artificial Sequence
  nucleotide sequence of nucleotide sequence of VEGF binder-hu IgG1 Fc DANG-hu CRIg
tccgatactggcagacccttcgtcgagatgtacagcgagattcctgagatcatccacatgacagagggacgggaactggtgattccttgcagagtgacatctccaaacatcacagtgaccctgaagaagtttcctctggacaccctgatccctgacggcaagcgcatcatctgggacagcagaaagggattcatcatcagcaacgccacctacaaggaaatcggcctcctgacctgcgaggccaccgtgaacggacacctgtataaaaccaattacctgacacaccggcaaacaaacaccatcatcgacgtggtgctgagccctagccacggcatcgagctgagcgtgggcgagaagctggtgctgaactgcaccgccagaaccgaactgaacgtgggcatcgatttcaactgggaatacccctcctctaagcaccagcataagaaactggttaatagagatctgaaaacccagagcggcagcgaaatgaaaaagttcctgtctacactgaccatcgacggcgtgaccagaagcgaccagggcctgtacacctgtgccgcttctagcggcctgatgaccaagaagaacagcacattcgtgcgggtgcacgagaagggaggaggcggcagcgataagacccacacatgcccaccctgtcctgcaccagagctgctgggaggaccatccgtgttcctgtttcctccaaagcctaaggacaccctgatgatctctcggaccccagaggtgacatgcgtggtggtggccgtgagccacgaggaccccgaggtgaagtttaactggtacgtggatggcgtggaggtgcacaatgccaagaccaagccccgggaggagcagtacggctccacctatagagtggtgtctgtgctgacagtgctgcaccaggattggctgaacggcaaggagtataagtgcaaggtgtccaataaggccctgcccgcccctatcgagaagaccatctctaaggcaaagggacagccaagggagccacaggtgtacacactgcccccttccagagacgagctgaccaagaaccaggtgtctctgacatgtctggtgaagggcttctatccctctgatatcgccgtggagtgggagagcaatggccagcctgagaacaattacaagaccacaccacccgtgctggactccgatggctctttctttctgtatagcaagctgaccgtggataagtccagatggcagcagggcaacgtgttttcttgtagcgtgatgcacgaggccctgcacaatcactacacacagaagtccctgtctctgagccccggcggaggtggcggttctgggggaggcggaagccggcctatcctggaggtgccagagtccgtgaccggaccatggaagggcgacgtgaacctgccctgcacctacgatcctctgcagggctatacacaggtgctggtgaagtggctggtgcagaggggcagcgaccctgtgaccatcttcctgcgcgacagctccggcgatcacatccagcaggccaagtaccagggcaggctgcacgtgtctcacaaggtgcctggcgatgtgagcctgcagctgtccaccctggagatggacgatcgcagccactatacatgtgaggtgacctggcagacaccagacggcaatcaggtggtgcgggataagatcaccgagctgagagtgcagaagctgtccgtgtctaagccaaccgtgaccacaggcagcggctacggcttcacagtgccccagggcatgaggatctccctgcagtgccaggcaaggggctctccacctatcagctacatctggtataagcagcagaccaacaatcaggagcctatcaaggtggccaccctgtccacactgctgttcaagccagccgtgatcgccgacagcggctcctatttttgtacagcaaagggacaagtgggctccgagcagcactctgacatcgtgaagtttgtggtgaaggattctagcaagctgctgaagaccaagacagaggcccctaccacaatgacctacccactgaaggccaccagcacagtgaagcagtcctgggactggaccacagacatggatggctatctgggcgagacatctgccggaccaggcaagagcctgccagga

SEQ ID NO: 27 - DNA, 1308 bp, Artificial Sequence
  nucleotide sequence of VEGF binder-hu IgG1 Fc DANG
tccgatactggcagacccttcgtcgagatgtacagcgagattcctgagatcatccacatgacagagggacgggaactggtgattccttgcagagtgacatctccaaacatcacagtgaccctgaagaagtttcctctggacaccctgatccctgacggcaagcgcatcatctgggacagcagaaagggattcatcatcagcaacgccacctacaaggaaatcggcctcctgacctgcgaggccaccgtgaacggacacctgtataaaaccaattacctgacacaccggcaaacaaacaccatcatcgacgtggtgctgagccctagccacggcatcgagctgagcgtgggcgagaagctggtgctgaactgcaccgccagaaccgaactgaacgtgggcatcgatttcaactgggaatacccctcctctaagcaccagcataagaaactggttaatagagatctgaaaacccagagcggcagcgaaatgaaaaagttcctgtctacactgaccatcgacggcgtgaccagaagcgaccagggcctgtacacctgtgccgcttctagcggcctgatgaccaagaagaacagcacattcgtgcgggtgcacgagaagggaggaggcggcagcgataagacccacacatgcccaccctgtcctgcaccagagctgctgggaggaccatccgtgttcctgtttcctccaaagcctaaggacaccctgatgatctctcggaccccagaggtgacatgcgtggtggtggccgtgagccacgaggaccccgaggtgaagtttaactggtacgtggatggcgtggaggtgcacaatgccaagaccaagccccgggaggagcagtacggctccacctatagagtggtgtctgtgctgacagtgctgcaccaggattggctgaacggcaaggagtataagtgcaaggtgtccaataaggccctgcccgcccctatcgagaagaccatctctaaggcaaagggacagccaagggagccacaggtgtacacactgcccccttccagagacgagctgaccaagaaccaggtgtctctgacatgtctggtgaagggcttctatccctctgatatcgccgtggagtgggagagcaatggccagcctgagaacaattacaagaccacaccacccgtgctggactccgatggctctttctttctgtatagcaagctgaccgtggataagtccagatggcagcagggcaacgtgttttcttgtagcgtgatgcacgaggccctgcacaatcactacacacagaagtccctgtctctgagccccggc

SEQ ID NO: 28 - DNA, 624 bp, Artificial Sequence
  nucleotide sequence of hu IgG1 Fc DANG
tccgtgttcctgtttccacccaagcccaaggataccctgatgatcagcaggaccccagaggtgacatgcgtggtggtggccgtgtcccacgaggaccctgaggtgaagttcaactggtacgtggatggcgtggaggtgcacaatgccaagaccaagccacgggaggagcagtacggctccacctatagagtggtgtctgtgctgacagtgctgcaccaggactggctgaacggcaaggagtataagtgcaaggtgtctaataaggccctgcctgccccaatcgagaagaccatcagcaaggcaaagggacagccaagggagcctcaggtgtacacactgcctccatcccgcgacgagctgaccaagaaccaggtgtctctgacatgtctggtgaagggcttctatccttctgatatcgccgtggagtgggagagcaatggccagccagagaacaattacaagaccacaccccctgtgctggactctgatggcagcttctttctgtatagcaagctgaccgtggataagtccaggtggcagcagggcaacgtgtttagctgttccgtgatgcacgaggccctgcacaatcactacacacagaagtctctgagcctgtcccctggc

SEQ ID NO: 29 - DNA, 1221 bp, Artificial Sequence
  nucleotide sequence of mu CRIg-mu IgG2a Fc DANG
caccctacactgaagacacccgagtccgtcaccggcacatggaagggagacgtcaagatccagtgcatctacgaccccctcagaggctatagacaagtgctcgtcaaatggctcgtgagacacggctccgatagcgtgaccatctttctgagagacagcaccggcgaccatatccagcaagccaagtatagaggcagactgaaggtgagccacaaggtgcccggcgatgtgtctctgcagatcaacacactgcagatggatgatagaaaccactatacatgcgaggtcacatggcagacccccgatggaaaccaagtgattagagacaagatcatcgagctgagggtgaggaagtacaacccccctaggatcaacaccgaggctcctaccacactgcacagctctctggaggccacaacaatcatgtccagcaccagcgatctgacaaccaacggaaccggcaagctggaagagaccatcgccggcagcggaaggaatctgcccggcggaggaggcagcgagcctagaggacccacaattaagccttgccccccttgcaaatgtcccgcccctaatctgctcggcggccccagcgtgttcatcttcccccccaagattaaggacgtgctgatgatctctctgtcccccattgtgacatgcgtggtcgtggctgtctccgaggacgaccccgacgtccagatcagctggttcgtcaacaatgtggaggtccataccgcccagacacagacccatagagaggattacggcagcacactgagagtggtcagcgctctgcccatccaacaccaagactggatgagcggcaaggagttcaagtgtaaagtgaacaacaaggatctgcccgcccccattgagaggaccatctccaaacctaagggcagcgtgagggctcctcaagtgtatgtgctccccccccccgaggaggaaatgaccaagaagcaagtgacactgacatgcatggtcaccgacttcatgcccgaggacatctacgtggagtggaccaacaacggcaagaccgagctgaattacaagaacaccgaacccgtgctggatagcgatggctcctacttcatgtacagcaagctgagagtggagaaaaagaactgggtcgagaggaacagctacagctgctccgtcgtgcatgagggcctccacaaccaccatacaaccaagagcttctctaggacacccggcaaatga

SEQ ID NO: 30 - DNA, 1863 bp, Artificial Sequence
  nucleotide sequence of mu CRIg-mu IgG2a Fc DANG-VEGF binder
caccctacactgaagacacccgagtccgtcaccggcacatggaagggagacgtcaagatccagtgcatctacgaccccctcagaggctatagacaagtgctcgtcaaatggctcgtgagacacggctccgatagcgtgaccatctttctgagagacagcaccggcgaccatatccagcaagccaagtatagaggcagactgaaggtgagccacaaggtgcccggcgatgtgtctctgcagatcaacacactgcagatggatgatagaaaccactatacatgcgaggtcacatggcagacccccgatggaaaccaagtgattagagacaagatcatcgagctgagggtgaggaagtacaacccccctaggatcaacaccgaggctcctaccacactgcacagctctctggaggccacaacaatcatgtccagcaccagcgatctgacaaccaacggaaccggcaagctggaagagaccatcgccggcagcggaaggaatctgcccggcggaggaggcagcgagcctagaggacccacaattaagccttgccccccttgcaaatgtcccgcccctaatctgctcggcggccccagcgtgttcatcttcccccccaagattaaggacgtgctgatgatctctctgtcccccattgtgacatgcgtggtcgtggctgtctccgaggacgaccccgacgtccagatcagctggttcgtcaacaatgtggaggtccataccgcccagacacagacccatagagaggattacggcagcacactgagagtggtcagcgctctgcccatccaacaccaagactggatgagcggcaaggagttcaagtgtaaagtgaacaacaaggatctgcccgcccccattgagaggaccatctccaaacctaagggcagcgtgagggctcctcaagtgtatgtgctccccccccccgaggaggaaatgaccaagaagcaagtgacactgacatgcatggtcaccgacttcatgcccgaggacatctacgtggagtggaccaacaacggcaagaccgagctgaattacaagaacaccgaacccgtgctggatagcgatggctcctacttcatgtacagcaagctgagagtggagaaaaagaactgggtcgagaggaacagctacagctgctccgtcgtgcatgagggcctccacaaccaccatacaaccaagagcttctctaggacacccggcggcggaggcggatccggaggaggcggcagctccgataccggaagacctttcgtggagatgtattccgagattcccgagatcatccacatgaccgagggaagagagctggtcatcccttgtagagtcacaagccccaacattaccgtgaccctcaagaagttccctctggacacactgattcccgacggcaagaggattatctgggactctaggaagggcttcatcatcagcaacgccacctataaagagatcggactgctgacatgcgaggccacagtgaatggccacctctacaagaccaactatctgacccatagacaaaccaacaccattatcgacgtggtgctgagccctagccacggcatcgaactcagcgtgggagagaaactggtgctgaattgcaccgctaggaccgaactcaacgtgggaatcgacttcaactgggagtacccctccagcaagcaccagcacaagaagctcgtgaatagagatctgaagacccagagcggaagcgagatgaagaaattcctctccacactgaccatcgatggcgtgacaaggagcgaccaaggactgtacacatgcgctgcttccagcggactgatgacaaagaagaacagcaccttcgtgagggtccacgaaaaatga

SEQ ID NO: 31 - DNA, 1233 bp, Artificial Sequence
  nucleotide sequence of mu IgG2a Fc DANG-mu CRIg
gagcctagaggcccaacaatcaagccttgtcctccttgcaaatgccctgctcctaacctgctgggcggccctagcgtctttatcttccctcctaagatcaaagacgtgctgatgatcagcctgagccctatcgtgacctgcgtggtggtggccgtgtctgaggacgatcctgacgtgcagatcagctggttcgtgaacaatgtggaagtgcacacagcccagacacaaacacacagagaggattacggcagcacactgcgcgtggtttccgccctgccaatccagcaccaggactggatgagcggcaaggaattcaagtgcaaagtgaacaacaaggacctgcctgcccctatcgagagaaccattagcaagcccaagggatcagttagagcccctcaggtgtacgtgctgcccccccccgaggaggaaatgaccaaaaagcaggtgaccctgacatgcatggtgactgacttcatgcctgaggacatctacgtggaatggaccaacaacggaaagaccgagctcaactacaagaacaccgagcccgtgcttgattctgacggcagctacttcatgtacagcaagctgcgggtggaaaagaagaactgggtggaaagaaatagctatagctgttctgtggtgcacgagggcctgcataatcaccacaccaccaagtccttcagccggacccctggcggcggcggaggatccggcggaggcgggagccaccccaccctgaaaacccccgagagcgtgacaggaacatggaagggcgatgtcaagatccaatgtatctacgaccccctgagaggctacagacaggtgctggtgaagtggctggtcaggcacggcagcgacagcgtgaccatctttctgcgggactctacaggagatcacatccagcaggccaagtaccggggcagactgaaggtctcccacaaggtgcctggcgacgtgtccctgcagatcaacacactgcagatggatgacagaaaccactacacctgcgaggtgacctggcagacccctgatggcaaccaggtgatcagagataagatcatcgagctgcgggtgcggaagtacaaccccccgcggatcaacaccgaggccccaaccaccctccattctagcctggaagctacaaccatcatgagcagcaccagcgacctgaccaccaatggcacaggcaagctggaagagacaatcgccggctctggcagaaacctgcctggc

SEQ ID NO: 32 - DNA, 1863 bp, Artificial Sequence
  nucleotide sequence of VEGF binder-mu IgG2a Fc DANG-mu CRIg
tccgatactggcagacccttcgtcgagatgtacagcgagattcctgagatcatccacatgacagagggacgggaactggtgattccttgcagagtgacatctccaaacatcacagtgaccctgaagaagtttcctctggacaccctgatccctgacggcaagcgcatcatctgggacagcagaaagggattcatcatcagcaacgccacctacaaggaaatcggcctcctgacctgcgaggccaccgtgaacggacacctgtataaaaccaattacctgacacaccggcaaacaaacaccatcatcgacgtggtgctgagccctagccacggcatcgagctgagcgtgggcgagaagctggtgctgaactgcaccgccagaaccgaactgaacgtgggcatcgatttcaactgggaatacccctcctctaagcaccagcataagaaactggttaatagagatctgaaaacccagagcggcagcgaaatgaaaaagttcctgtctacactgaccatcgacggcgtgaccagaagcgaccagggcctgtacacctgtgccgcttctagcggcctgatgaccaagaagaacagcacattcgtgcgggtgcacgagaagggcggcggaggtagcgagcctagaggcccaacaatcaagccttgtcctccttgcaaatgccctgctcctaacctgctgggcggccctagcgtctttatcttccctcctaagatcaaagacgtgctgatgatcagcctgagccctatcgtgacctgcgtggtggtggccgtgtctgaggacgatcctgacgtgcagatcagctggttcgtgaacaatgtggaagtgcacacagcccagacacaaacacacagagaggattacggcagcacactgcgcgtggtttccgccctgccaatccagcaccaggactggatgagcggcaaggaattcaagtgcaaagtgaacaacaaggacctgcctgcccctatcgagagaaccattagcaagcccaagggatcagttagagcccctcaggtgtacgtgctgcccccccccgaggaggaaatgaccaaaaagcaggtgaccctgacatgcatggtgactgacttcatgcctgaggacatctacgtggaatggaccaacaacggaaagaccgagctcaactacaagaacaccgagcccgtgcttgattctgacggcagctacttcatgtacagcaagctgcgggtggaaaagaagaactgggtggaaagaaatagctatagctgttctgtggtgcacgagggcctgcataatcaccacaccaccaagtccttcagccggacccctggcggcggcggaggatccggcggaggcgggagccaccccaccctgaaaacccccgagagcgtgacaggaacatggaagggcgatgtcaagatccaatgtatctacgaccccctgagaggctacagacaggtgctggtgaagtggctggtcaggcacggcagcgacagcgtgaccatctttctgcgggactctacaggagatcacatccagcaggccaagtaccggggcagactgaaggtctcccacaaggtgcctggcgacgtgtccctgcagatcaacacactgcagatggatgacagaaaccactacacctgcgaggtgacctggcagacccctgatggcaaccaggtgatcagagataagatcatcgagctgcgggtgcggaagtacaaccccccgcggatcaacaccgaggccccaaccaccctccattctagcctggaagctacaaccatcatgagcagcaccagcgacctgaccaccaatggcacaggcaagctggaagagacaatcgccggctctggcagaaacctgcctggc

SEQ ID NO: 33 - DNA, 654 bp, Artificial Sequence
  nucleotide sequence of mu IgG2a Fc DANG
gcccccaatctgctgggaggcccttccgtcttcatcttcccccccaagatcaaggacgtgctgatgatctctctgagccccatcgtgacatgcgtggtggtggccgtgagcgaggacgatcccgacgtgcagatcagctggttcgtcaacaacgtggaggtgcataccgcccaaacacagacccatagagaggactacggctccacactgagagtggtgtccgctctgcccatccagcatcaagactggatgagcggcaaggagttcaagtgcaaggtgaacaacaaggatctgcccgcccctatcgagaggaccatctccaagcccaaaggctccgtgagagctccccaagtgtatgtgctgcctccccccgaggaggagatgaccaagaagcaagtgacactgacatgcatggtgaccgatttcatgcccgaagacatctacgtggagtggaccaacaacggcaagaccgagctcaactacaagaacaccgagcccgtgctcgacagcgacggcagctacttcatgtacagcaagctgagggtcgagaagaaaaactgggtggagaggaacagctacagctgtagcgtggtgcacgagggactgcacaaccaccataccaccaagagcttctccagaacacccggcaagtga

SEQ ID NO: 34 - DNA, 1344 bp, Artificial Sequence
  nucleotide sequence of mu IgG2a Fc DANG-VEGF binder
gagcctagaggacccacaattaagccttgccccccttgcaaatgtcccgcccctaatctgctcggcggccccagcgtgttcatcttcccccccaagattaaggacgtgctgatgatctctctgtcccccattgtgacatgcgtggtcgtggctgtctccgaggacgaccccgacgtccagatcagctggttcgtcaacaatgtggaggtccataccgcccagacacagacccatagagaggattacggcagcacactgagagtggtcagcgctctgcccatccaacaccaagactggatgagcggcaaggagttcaagtgtaaagtgaacaacaaggatctgcccgcccccattgagaggaccatctccaaacctaagggcagcgtgagggctcctcaagtgtatgtgctccccccccccgaggaggaaatgaccaagaagcaagtgacactgacatgcatggtcaccgacttcatgcccgaggacatctacgtggagtggaccaacaacggcaagaccgagctgaattacaagaacaccgaacccgtgctggatagcgatggctcctacttcatgtacagcaagctgagagtggagaaaaagaactgggtcgagaggaacagctacagctgctccgtcgtgcatgagggcctccacaaccaccatacaaccaagagcttctctaggacacccggcggcggaggcggatccggaggaggcggcagctccgataccggaagacctttcgtggagatgtattccgagattcccgagatcatccacatgaccgagggaagagagctggtcatcccttgtagagtcacaagccccaacattaccgtgaccctcaagaagttccctctggacacactgattcccgacggcaagaggattatctgggactctaggaagggcttcatcatcagcaacgccacctataaagagatcggactgctgacatgcgaggccacagtgaatggccacctctacaagaccaactatctgacccatagacaaaccaacaccattatcgacgtggtgctgagccctagccacggcatcgaactcagcgtgggagagaaactggtgctgaattgcaccgctaggaccgaactcaacgtgggaatcgacttcaactgggagtacccctccagcaagcaccagcacaagaagctcgtgaatagagatctgaagacccagagcggaagcgagatgaagaaattcctctccacactgaccatcgatggcgtgacaaggagcgaccaaggactgtacacatgcgctgcttccagcggactgatgacaaagaagaacagcaccttcgtgagggtccacgaaaaatga

SEQ ID NO: 35 - DNA, 1293 bp, Artificial Sequence
  nucleotide sequence of Aflibercept
tccgatactggcagacccttcgtcgagatgtacagcgagattcctgagatcatccacatgacagagggacgggaactggtgattccttgcagagtgacatctccaaacatcacagtgaccctgaagaagtttcctctggacaccctgatccctgacggcaagcgcatcatctgggacagcagaaagggattcatcatcagcaacgccacctacaaggaaatcggcctcctgacctgcgaggccaccgtgaacggacacctgtataaaaccaattacctgacacaccggcaaacaaacaccatcatcgacgtggtgctgagccctagccacggcatcgagctgagcgtgggcgagaagctggtgctgaactgcaccgccagaaccgaactgaacgtgggcatcgatttcaactgggaatacccctcctctaagcaccagcataagaaactggttaatagagatctgaaaacccagagcggcagcgaaatgaaaaagttcctgtctacactgaccatcgacggcgtgaccagaagcgaccagggcctgtacacctgtgccgcttctagcggcctgatgaccaagaagaacagcacattcgtgcgggtgcacgagaaggacaaaactcacacatgcccaccgtgcccagcacctgaactcctggggggaccgtcagtcttcctcttccccccaaaacccaaggacaccctcatgatctcccggacccctgaggtcacatgcgtggtggtggacgtgagccacgaagaccctgaggtcaagttcaactggtacgtggacggcgtggaggtgcataatgccaagacaaagccgcgggaggagcagtacaacagcacgtaccgtgtggtcagcgtcctcaccgtcctgcaccaggactggctgaatggcaaggagtacaagtgcaaggtctccaacaaagccctcccagcccccatcgagaaaaccatctccaaagccaaagggcagccccgagaaccacaggtgtacaccctgcccccatcccgggatgagctgaccaagaaccaggtcagcctgacctgcctggtcaaaggcttctatcccagcgacatcgccgtggagtgggagagcaatgggcagccggagaacaactacaagaccacgcctcccgtgctggactccgacggctccttcttcctctacagcaagctcaccgtggacaagagcaggtggcagcaggggaacgtcttctcatgctccgtgatgcatgaggctctgcacaaccactacacgcagaagagcctctccctgtctccgggt

SEQ ID NO: 36 - protein, 453 aa, Artificial Sequence
  Heavy chain of anti-VEGF antibody Bevacizumab
EVQLVESGGGLVQPGGSLRLSCAASGYTFTNYGMNWVRQAPGKGLEWVGWINTYTGEPTYAADFKRRFTFSLDTSKSTAYLQMNSLRAEDTAVYYCAKYPHYYGSSHWYFDVWGQGTLVTVSSASTKGPSVFPLAPSSKSTSGGTAALGCLVKDYFPEPVTVSWNSGALTSGVHTFPAVLQSSGLYSLSSVVTVPSSSLGTQTYICNVNHKPSNTKVDKKVEPKSCDKTHTCPPCPAPELLGGPSVFLFPPKPKDTLMISRTPEVTCVVVDVSHEDPEVKFNWYVDGVEVHNAKTKPREEQYNSTYRVVSVLTVLHQDWLNGKEYKCKVSNKALPAPIEKTISKAKGQPREPQVYTLPPSREEMTKNQVSLTCLVKGFYPSDIAVEWESNGQPENNYKTTPPVLDSDGSFFLYSKLTVDKSRWQQGNVFSCSVMHEALHNHYTQKSLSLSPGK

SEQ ID NO: 37 - protein, 214 aa, Artificial Sequence
  Light chain of anti-VEGF antibody Bevacizumab
DIQMTQSPSSLSASVGDRVTITCSASQDISNYLNWYQQKPGKAPKVLIYFTSSLHSGVPSRFSGSGSGTDFTLTISSLQPEDFATYYCQQYSTVPWTFGQGTKVEIKRTVAAPSVFIFPPSDEQLKSGTASVVCLLNNFYPREAKVQWKVDNALQSGNSQESVTEQDSKDSTYSLSSTLTLSKADYEKHKVYACEVTHQGLSSPVTKSFNRGEC

SEQ ID NO: 38 - protein, 231 aa, Artificial Sequence
  Variable Heavy chain of anti-VEGF antibody Ranibizumab
EVQLVESGGGLVQPGGSLRLSCAASGYDFTHYGMNWVRQAPGKGLEWVGWINTYTGEPTYAADFKRRFTFSLDTSKSTAYLQMNSLRAEDTAVYYCAKYPYYYGTSHWYFDVWGQGTLVTVSSASTKGPSVFPLAPSSKSTSGGTAALGCLVKDYFPEPVTVSWNSGALTSGVHTFPAVLQSSGLYSLSSVVTVPSSSLGTQTYICNVNHKPSNTKVDKKVEPKSCDKTHL

SEQ ID NO: 39 - protein, 214 aa, Artificial Sequence
  Light chain of anti-VEGF antibody Ranibizumab
DIQLTQSPSSLSASVGDRVTITCSASQDISNYLNWYQQKPGKAPKVLIYFTSSLHSGVPSRFSGSGSGTDFTLTISSLQPEDFATYYCQQYSTVPWTFGQGTKVEIKRTVAAPSVFIFPPSDEQLKSGTASVVCLLNNFYPREAKVQWKVDNALQSGNSQESVTEQDSKDSTYSLSSTLTLSKADYEKHKVYACEVTHQGLSSPVTKSFNRGEC

SEQ ID NO: 40 - protein, 446 aa, Artificial Sequence
  Heavy chain of anti-VEGF antibody Ramucirumab
EVQLVQSGGGLVKPGGSLRLSCAASGFTFSSYSMNWVRQAPGKGLEWVSSISSSSSYIYYADSVKGRFTISRDNAKNSLYLQMNSLRAEDTAVYYCARVTDAFDIWGQGTMVTVSSASTKGPSVFPLAPSSKSTSGGTAALGCLVKDYFPEPVTVSWNSGALTSGVHTFPAVLQSSGLYSLSSVVTVPSSSLGTQTYICNVNHKPSNTKVDKKVEPKSCDKTHTCPPCPAPELLGGPSVFLFPPKPKDTLMISRTPEVTCVVVDVSHEDPEVKFNWYVDGVEVHNAKTKPREEQYNSTYRVVSVLTVLHQDWLNGKEYKCKVSNKALPAPIEKTISKAKGQPREPQVYTLPPSREEMTKNQVSLTCLVKGFYPSDIAVEWESNGQPENNYKTTPPVLDSDGSFFLYSKLTVDKSRWQQGNVFSCSVMHEALHNHYTQKSLSLSPGK

SEQ ID NO: 41 - protein, 214 aa, Artificial Sequence
  Light chain of anti-VEGF antibody Ramucirumab
DIQMTQSPSSVSASIGDRVTITCRASQGIDNWLGWYQQKPGKAPKLLIYDASNLDTGVPSRFSGSGSGTYFTLTISSLQAEDFAVYFCQQAKAFPPTFGGGTKVDIKGTVAAPSVFIFPPSDEQLKSGTASVVCLLNNFYPREAKVQWKVDNALQSGNSQESVTEQDSKDSTYSLSSTLTLSKADYEKHKVYACEVTHQGLSSPVTKSFNRGEC

SEQ ID NO: 42 - protein, 252 aa, Artificial Sequence
  scFv of anti-VEGF antibody Brolucizumab (VL-linker-VL)
MEIVMTQSPSTLSASVGDRVIITCQASEIIHSWLAWYQQKPGKAPKLLIYLASTLASGVPSRFSGSGSGAEFTLTISSLQPDDFATYYCQNVYLASTNGANFGQGTKLTVLGGGGGSGGGGSGGGGSGGGGSEVQLVESGGGLVQPGGSLRLSCTASGFSLTDYYYMTWVRQAPGKGLEWVGFIDPDDDPYYATWAKGRFTISRDNSKNTLYLQMNSLRAEDTAVYYCAGGDHNSGWGLDIWGQGTLVTVSS

SEQ ID NO: 43 - protein, 453 aa, Artificial Sequence
  Heavy chain of anti-VEGF antibody Faricimab
EVQLVESGGGLVQPGGSLRLSCAASGYDFTHYGMNWVRQAPGKGLEWVGWINTYTGEPTYAADFKRRFTFSLDTSKSTAYLQMNSLRAEDTAVYYCAKYPYYYGTSHWYFDVWGQGTLVTVSSASTKGPSVFPLAPSSKSTSGGTAALGCLVKDYFPEPVTVSWNSGALTSGVHTFPAVLQSSGLYSLSSVVTVPSSSLGTQTYICNVNHKPSNTKVDKKVEPKSCDKTHTCPPCPAPEAAGGPSVFLFPPKPKDTLMASRTPEVTCVVVDVSHEDPEVKFNWYVDGVEVHNAKTKPREEQYNSTYRVVSVLTVLAQDWLNGKEYKCKVSNKALGAPIEKTISKAKGQPREPQVYTLPPCRDELTKNQVSLWCLVKGFYPSDIAVEWESNGQPENNYKTTPPVLDSDGSFFLYSKLTVDKSRWQQGNVFSCSVMHEALHNAYTQKSLSLSPGK

SEQ ID NO: 44 - protein, 214 aa, Artificial Sequence; identical to SEQ ID NO: 39
  Light chain of anti-VEGF antibody Faricimab

SEQ ID NO: 45 - protein, 453 aa, Artificial Sequence
  Heavy chain of anti-VEGF antibody KSI-301
EVQLVESGGGLVQPGGSLRLSCAASGYDFTHYGMNWVRQAPGKGLEWVGWINTYTGEPTYAADFKRRFTFSLDTSKSTAYLQMNSLRAEDTAVYYCAKYPYYYGTSHWYFDVWGQGTLVTVSSASTKGPSVFPLAPSSKSTSGGTAALGCLVKDYFPEPVTVSWNSGALTSGVHTFPAVLQSSGLYSLSSVVTVPSSSLGTQTYICNVNHKPSNTKVDKKVEPKSCDKTHTCPPCPAPEAAGAPSVFLFPPKPKDTLMISRTPEVTCVVVDVSHEDPEVKFNWYVDGVEVHNAKTKPREEQYNSTYRVVSVLTVLHQDWLNGKEYKCKVSNKALPAPIEKTISKAKGQPREPQVYTLPPSREEMTKNQVSLTCLVKGFYPSDIAVEWESNGQPENNYKTTPPVLDSDGSFFLYSKLTVDKSRWQQGNVFSCSVMHEALHNHYTQKSLSCSPGK

SEQ ID NO: 46 - protein, 214 aa, Artificial Sequence; identical to SEQ ID NO: 39
  Light chain of anti-VEGF antibody KSI-301

SEQ ID NO: 47 - protein, 453 aa, Artificial Sequence
  Heavy chain of anti-VEGF antibody Vanucizumab
EVQLVESGGGLVQPGGSLRLSCAASGYTFTNYGMNWVRQAPGKGLEWVGWINTYTGEPTYAADFKRRFTFSLDTSKSTAYLQMNSLRAEDTAVYYCAKYPHYYGSSHWYFDVWGQGTLVTVSSASTKGPSVFPLAPSSKSTSGGTAALGCLVKDYFPEPVTVSWNSGALTSGVHTFPAVLQSSGLYSLSSVVTVPSSSLGTQTYICNVNHKPSNTKVDKKVEPKSCDKTHTCPPCPAPELLGGPSVFLFPPKPKDTLMISRTPEVTCVVVDVSHEDPEVKFNWYVDGVEVHNAKTKPREEQYNSTYRVVSVLTVLHQDWLNGKEYKCKVSNKALPAPIEKTISKAKGQPREPQVYTLPPCRDELTKNQVSLWCLVKGFYPSDIAVEWESNGQPENNYKTTPPVLDSDGSFFLYSKLTVDKSRWQQGNVFSCSVMHEALHNHYTQKSLSLSPGK

SEQ ID NO: 48 - protein, 214 aa, Artificial Sequence; identical to SEQ ID NO: 37
  Light chain of anti-VEGF antibody Vanucizumab

SEQ ID NO: 49 - protein, 5 aa, Artificial Sequence
  CDR1 of anti-VEGF VHH-antibody BI-836880
SYSMG

SEQ ID NO: 50 - protein, 16 aa, Artificial Sequence
  CDR2 of anti-VEGF VHH-antibody BI-836880
AISKGGYKYDAVSLEG

SEQ ID NO: 51 - protein, 17 aa, Artificial Sequence
  CDR3 of anti-VEGF VHH-antibody BI-836880
SRAYGSSRLRLADTYEY

SEQ ID NO: 52 - protein, 11 aa, Artificial Sequence
  HC-CDR1 of HuMab G6-31
SASQDISNYLN

SEQ ID NO: 53 - protein, 16 aa, Artificial Sequence
  HC-CDR2 of HuMab G6-31
GITPAGGYTYYADSVK

SEQ ID NO: 54 - protein, 5 aa, Artificial Sequence
  HC-CDR3 of HuMab G6-31
DYWIH

SEQ ID NO: 55 - protein, 9 aa, Artificial Sequence
  LC-CDR1 of HuMab G6-31
QQGYGNPFT

SEQ ID NO: 56 - protein, 7 aa, Artificial Sequence
  LC-CDR2 of HuMab G6-31
SASFLYS

SEQ ID NO: 57 - protein, 11 aa, Artificial Sequence
  LC-CDR3 of HuMab G6-31
RASQDVSTAVA

SEQ ID NO: 58 - protein, 12 aa, Artificial Sequence
  HC-CDR1 of B20-4.1
WGHSTSPWAMDY

SEQ ID NO: 59 - protein, 16 aa, Artificial Sequence
  HC-CDR2 of B20-4.1
AIWPFGGYTHYADSVK

SEQ ID NO: 60 - protein, 8 aa, Artificial Sequence
  HC-CDR3 of B20-4.1
FSINGSWI

SEQ ID NO: 61 - protein, 9 aa, Artificial Sequence
  LC-CDR1 of B20-4.1
QQSNTSPLT

SEQ ID NO: 62 - protein, 8 aa, Artificial Sequence
  LC-CDR2 of B20-4.1
YAASNLAS

SEQ ID NO: 63 - protein, 11 aa, Artificial Sequence
  LC-CDR3 of B20-4.1
RASQVIRRSLA

SEQ ID NO: 64 - protein, 453 aa, Artificial Sequence
  Heavy chain of BAT-5906
EVQLVESGGGLVQPGGSLRLSCAASGYDFTHYGMNWVRQAPGKGLEWVWINTYTGEPTYAADFKRRFTFSLDTSKSTAYLQMNSLRAEDTAVYYCAKYPYYYGTSHWYFDVWGQGTLVTVSSASTKGPSVFPLAPSSKSTSGGTAALGCLVKDYFPEPVTVSWNSGALTSGVHTFPAVLQSSGLYSLSSVVTVPSSSLGTQTYICNVNIIKPSNTKVDKKVEPKSCDKTHTCPPCPAPELLGGPSVFLFPPKPKDTLMISRTPEVTCVVVDVSHEDPEVKFNWYVDGVEVHNAKTKPREEQYNSTYRVVSVLTVLHQDWLNGKEYKCKVSNKALPAPIEKTISKAKGQPREPQVYTLPPSREEMTKNQVSLTCLVKGFYPSDIAVEWESNGQPENNYKTTPPVLDSDGSFFLYSKLTVDKSRWQQGNVFSCSVMHEALHNHYTQKSLSLSPGK

SEQ ID NO: 65 - protein, 214 aa, Artificial Sequence; identical to SEQ ID NO: 39
  Light chain of BAT-5906

SEQ ID NO: 66 - protein, 447 aa, Artificial Sequence
  Heavy chain of Navicixizumab
QVQLVQSGAEVKKPGASVKVSCKASGYTFTNYWMHWVRQAPGQGLEWMGDINPSNGRTSYKEKFKRRVTLSVDKSSSTAYMELSSLRSEDTAVYFCTIHYDDKYYPLMDYWGQGTLVTVSSASTKGPSVFPLAPCSRSTSESTAALGCLVKDYFPEPVTVSWNSGALTSGVHTFPAVLQSSGLYSLSSVVTVPSSNFGTQTYTCNVDHKPSNTKVDKTVERKCCVECPPCPAPPVAGPSVFLFPPKPKDTLMISRTPEVTCVVVDVSHEDPEVQFNWYVDGVEVHNAKTKPREEQFNSTFRVVSVLTVVHQDWLNGKEYKCKVSNKGLPAPIEKTISKTKGQPREPQVYTLPPSREKMTKNQVSLTCLVKGFYPSDIAVEWESNGQPENNYKTTPPMLKSDGSFFLYSKLTVDKSRWQQGNVFSCSVMHEALHNHYTQKSLSLSPGK

SEQ ID NO: 67 - protein, 218 aa, Artificial Sequence
  Light chain of Navicixizumab
DIVMTQSPDSLAVSLGERATISCRASESVDNYGISFMKWFQQKPGQPPKLLIYAASNQGSGVPDRFSGSGSGTDFTLTISSLQAEDVAVYYCQQSKEVPWTFGGGTKVEIKRTVAAPSVFIFPPSDEQLKSGTASVVCLLNNFYPREAKVQWKVDNALQSGNSQESVTEQDSKDSTYSLSSTLTLSKADYEKHKVYACEVTHQGLSSPVTKSFNRGEC

SEQ ID NO: 68 - protein, 577 aa, Artificial Sequence
  Heavy chain of Dilpacimab
EVQLVESGGGLVQPGGSLRLSCAASGFTFSNFPMAWVRQAPGKGLEWVATISSSDGTTYYRDSVKGRFTISRDNAKNSLYLQMNSLRAEDTAVYYCARGYYNSPFAYWGQGTLVTVSSASTKGPEVQLVESGGGLVQPGGSLRLSCAASGYTFTNYGMNWVRQAPGKGLEWVGWINTYTGEPTYAADFKRRFTFSLDTSKSTAYLQMNSLRAEDTAVYYCAKYPHYYGSSHWYFDVWGQGTLVTVSSASTKGPSVFPLAPSSKSTSGGTAALGCLVKDYFPEPVTVSWNSGALTSGVHTFPAVLQSSGLYSLSSVVTVPSSSLGTQTYICNVNHKPSNTKVDKKVEPKSCDKTHTCPPCPAPEAAGGPSVFLFPPKPKDTLMISRTPEVTCVVVDVSHEDPEVKFNWYVDGVEVHNAKTKPREEQYNSTYRVVSVLTVLHQDWLNGKEYKCKVSNKALPAPIEKTISKAKGQPREPQVYTLPPSREEMTKNQVSLTCLVKGFYPSDIAVEWESNGQPENNYKTTPPVLDSDGSFFLYSKLTVDKSRWQQGNVFSCSVMHEALHNHYTQKSLSLSPGK

SEQ ID NO: 69 - protein, 334 aa, Artificial Sequence
  Light chain of Dilpacimab
DIQMTQSPSSLSASVGDRVTITCRASEDIYSNLAWYQQKPGKAPKLLIYDTNNLADGVPSRFSGSGSGTDFTLTISSLQPEDFATYYCQQYNNYPPTFGQGTKLEIKRTVAAPSVFIFPPDIQMTQSPSSLSASVGDRVTITCSASQDISNYLNWYQQKPGKAPKVLIYFTSSLHSGVPSRFSGSGSGTDFTLTISSLQPEDFATYYCQQYSTVPWTFGQGTKVEIKRTVAAPSVFIFPPSDEQLKSGTASVVCLLNNFYPREAKVQWKVDNALQSGNSQESVTEQDSKDSTYSLSSTLTLSKADYEKHKVYACEVTHQGLSSPVTKSFNRGEC

SEQ ID NO: 70 - protein, 116 aa, Artificial Sequence
  Heavy chain variable regions of hPV-19
DVQLVQSGVEVKNPGASVKVSCRASGYSFTNSGINWVKQAPGKGLKWMGWINTYTGEPTYADDFKGRFAFSLETSASSAYLQINNLKNEDTATYFCARFGDGYYWFFDVWGAGTTV

SEQ ID NO: 71 - protein, 113 aa, Artificial Sequence
  Light chain variable regions of hPV-19
DIVMTQSPDSLAVSLGERATINCKSSQSLLNSRTRKNFLAWYQQKPGQSPKLLIYWASTRESGVPDRFTGSGSGTDFTLTISSVQAEDLAVYYCKQSYNLYTFGGGTNLEIKR

SEQ ID NO: 72 - protein, 126 aa, Artificial Sequence
  Heavy chain variable regions of AT-001
QVQLVQSGAEVKKPGASVKVSCKASGGTFSSYAISWVRQAPGQGLEWMGGFDPEDGETIYAQKFQGRVTMTEDTSTDTAYMELSSLRSEDTAVYYCATGRSMVRGVIIPFNGMDVWGQGTTVTVSS

SEQ ID NO: 73 - protein, 107 aa, Artificial Sequence
  Light chain variable regions of AT-001
DIRMTQSPSSLSASVGDRVTITCRASQSISSYLNWYQQKPGKAPKLLIYAASSLQSGVPSRFSGSGSGTDFTLTISSLQPEDFATYYCQQSYSTPLTFGGGTKVEIK

SEQ ID NO: 74 - protein, 118 aa, Artificial Sequence
  amino sequences of human lg V of Crig
RPILEVPESVTGPWKGDVNLPCTYDPLQGYTQVLVKWLVQRGSDPVTIFLRDSSGDHIQQAKYQGRLHVSHKVPGDVSLQLSTLEMDDRSHYTCEVTWQTPDGNQVVRDKITELRVQK

SEQ ID NO: 75 - protein, 168 aa, Artificial Sequence
  Extracellular Domain of mouse CRIg
HPTLKTPESVTGTWKGDVKIQCIYDPLRGYRQVLVKWLVRHGSDSVTIFLRDSTGDHIQQAKYRGRLKVSHKVPGDVSLQINTLQMDDRNHYTCEVTWQTPDGNQVIRDKIIELRVRKYNPPRINTEAPTTLHSSLEATTIMSSTSDLTTNGTGKLEETIAGSGRNLP

SEQ ID NO: 76 - protein, 209 aa, Artificial Sequence
  Human IgG1 Fc DANG-K
SVFLFPPKPKDTLMISRTPEVTCVVVAVSHEDPEVKFNWYVDGVEVHNAKTKPREEQYGSTYRVVSVLTVLHQDWLNGKEYKCKVSNKALPAPIEKTISKAKGQPREPQVYTLPPSRDELTKNQVSLTCLVKGFYPSDIAVEWESNGQPENNYKTTPPVLDSDGSFFLYSKLTVDKSRWQQGNVFSCSVMHEALHNHYTQKSLSLSPGK

SEQ ID NO: 77 - protein, 118 aa, Artificial Sequence; identical to SEQ ID NO: 74
  HCDR1 of Bevacizumab

SEQ ID NO: 78 - protein, 17 aa, Artificial Sequence
  HCDR2 of Bevacizumab
WINTYTGEPTYAADFKR

SEQ ID NO: 79 - protein, 14 aa, Artificial Sequence
  HCDR3 of Bevacizumab
YPHYYGSSHWYFDV

SEQ ID NO: 80 - protein, 11 aa, Artificial Sequence
  LCDR1 of Bevacizumab
SASQDISNYLN

SEQ ID NO: 81 - protein, 7 aa, Artificial Sequence
  LCDR2 of Bevacizumab
FTSSLHS

SEQ ID NO: 82 - protein, 9 aa, Artificial Sequence
  LCDR3 of Bevacizumab
QQYSTVPWT

SEQ ID NO: 83 - protein, 10 aa, Artificial Sequence
  HCDR1 of Ranibizumab
GYDFTHYGMN

SEQ ID NO: 84 - protein, 17 aa, Artificial Sequence
  HCDR2 of Ranibizumab
WINTYTGEPTYAADFKR

SEQ ID NO: 85 - protein, 14 aa, Artificial Sequence
  HCDR3 of Ranibizumab
YPYYYGTSHWYFDV

SEQ ID NO: 86 - protein, 11 aa, Artificial Sequence
  LCDR1 of Ranibizumab
SASQDISNYLN

SEQ ID NO: 87 - protein, 7 aa, Artificial Sequence
  LCDR2 of Ranibizumab
FTSSLHS

SEQ ID NO: 88 - protein, 9 aa, Artificial Sequence
  LCDR3 of Ranibizumab
QQYSTVPWT

SEQ ID NO: 89 - protein, 10 aa, Artificial Sequence
  HCDR1 of Ramucirumab
GFTFSSYSMN

SEQ ID NO: 90 - protein, 17 aa, Artificial Sequence
  HCDR2 of Ramucirumab
SISSSSSYIYYADSVKG

SEQ ID NO: 91 - protein, 7 aa, Artificial Sequence
  HCDR3 of Ramucirumab
VTDAFDI

SEQ ID NO: 92 - protein, 11 aa, Artificial Sequence
  LCDR1 of Ramucirumab
RASQGIDNWLG

SEQ ID NO: 93 - protein, 7 aa, Artificial Sequence
  LCDR2 of Ramucirumab
DASNLDT

SEQ ID NO: 94 - protein, 9 aa, Artificial Sequence
  LCDR3 of Ramucirumab
QQAKAFPPT

SEQ ID NO: 95 - protein, 11 aa, Artificial Sequence
  CDR1 of Brolucizumab
QASEIIHSWLA

SEQ ID NO: 96 - protein, 7 aa, Artificial Sequence
  CDR2 of Brolucizumab
LASTLAS

SEQ ID NO: 97 - protein, 12 aa, Artificial Sequence
  CDR3 of Brolucizumab
QNVYLASTNGAN

SEQ ID NO: 98 - protein, 11 aa, Artificial Sequence
  CDR4 of Brolucizumab
GFSLTDYYYMT

SEQ ID NO: 99 - protein, 16 aa, Artificial Sequence
  CDR5 of Brolucizumab
FIDPDDDPYYATWAKG

SEQ ID NO: 100 - protein, 11 aa, Artificial Sequence
  CDR6 of Brolucizumab
GDHNSGWGLDI

SEQ ID NO: 101 - protein, 10 aa, Artificial Sequence
  HCDR1 of Faricimab
GYDFTHYGMN

SEQ ID NO: 102 - protein, 17 aa, Artificial Sequence
  HCDR2 of Faricimab
WINTYTGEPTYAADFKR

SEQ ID NO: 103 - protein, 14 aa, Artificial Sequence
  HCDR3 of Faricimab
YPYYYGTSHWYFDV

SEQ ID NO: 104 - protein, 11 aa, Artificial Sequence
  LCDR1 of Faricimab
SASQDISNYLN

SEQ ID NO: 105 - protein, 7 aa, Artificial Sequence
  LCDR2 of Faricimab
FTSSLHS

SEQ ID NO: 106 - protein, 9 aa, Artificial Sequence
  LCDR3 of Faricimab
QQYSTVPWT

SEQ ID NO: 107 - protein, 10 aa, Artificial Sequence
  HCDR1 of KSI-301
GYDFTHYGMN

SEQ ID NO: 108 - protein, 17 aa, Artificial Sequence
  HCDR2 of KSI-301
WINTYTGEPTYAADFKR

SEQ ID NO: 109 - protein, 14 aa, Artificial Sequence
  HCDR3 of KSI-301
YPYYYGTSHWYFDV

SEQ ID NO: 110 - protein, 11 aa, Artificial Sequence
  LCDR1 of KSI-301
SASQDISNYLN

SEQ ID NO: 111 - protein, 7 aa, Artificial Sequence
  LCDR2 of KSI-301
FTSSLHS

SEQ ID NO: 112 - protein, 9 aa, Artificial Sequence
  LCDR3 of KSI-301
QQYSTVPWT

SEQ ID NO: 113 - protein, 10 aa, Artificial Sequence
  HCDR1 of Vanucizumab
GYTFTNYGMN

SEQ ID NO: 114 - protein, 17 aa, Artificial Sequence
  HCDR2 of Vanucizumab
WINTYTGEPTYAADFKR

SEQ ID NO: 115 - protein, 14 aa, Artificial Sequence
  HCDR3 of Vanucizumab
YPHYYGSSHWYFDV

SEQ ID NO: 116 - protein, 11 aa, Artificial Sequence
  LCDR1 of Vanucizumab
SASQDISNYLN

SEQ ID NO: 117 - protein, 7 aa, Artificial Sequence
  LCDR2 of Vanucizumab
FTSSLHS

SEQ ID NO: 118 - protein, 9 aa, Artificial Sequence
  LCDR3 of Vanucizumab
QQYSTVPWT

SEQ ID NO: 119 - protein, 10 aa, Artificial Sequence
  HCDR1 of BAT-5906
GYDFTHYGMN

SEQ ID NO: 120 - protein, 17 aa, Artificial Sequence
  HCDR2 of BAT-5906
WINTYTGEPTYAADFKR

SEQ ID NO: 121 - protein, 14 aa, Artificial Sequence
  HCDR3 of BAT-5906
YPYYYGTSHWYFDV

SEQ ID NO: 122 - protein, 11 aa, Artificial Sequence
  LCDR1 of BAT-5906
SASQDISNYLN

SEQ ID NO: 123 - protein, 7 aa, Artificial Sequence
  LCDR2 of BAT-5906
FTSSLHS

SEQ ID NO: 124 - protein, 10 aa, Artificial Sequence
  LCDR3 of BAT-5906
CQQYSTVPWT

SEQ ID NO: 125 - protein, 5 aa, Artificial Sequence
  HCDR1 of Navicixizumab
NYWMH

SEQ ID NO: 126 - protein, 17 aa, Artificial Sequence
  HCDR2 of Navicixizumab
DINPSNGRTSYKEKFKR

SEQ ID NO: 127 - protein, 12 aa, Artificial Sequence
  HCDR3 of Navicixizumab
HYDDKYYPLMDY

SEQ ID NO: 128 - protein, 15 aa, Artificial Sequence
  LCDR1 of Navicixizumab
RASESVDNYGISFMK

SEQ ID NO: 129 - protein, 7 aa, Artificial Sequence
  LCDR2 of Navicixizumab
AASNQGS

SEQ ID NO: 130 - protein, 12 aa, Artificial Sequence
  LCDR3 of Navicixizumab
QQSKEVPWTFGG

SEQ ID NO: 131 - protein, 11 aa, Artificial Sequence
  HCDR1 of Dilpacimab
SGYTFTNYGMN

SEQ ID NO: 132 - protein, 16 aa, Artificial Sequence
  HCDR2 of Dilpacimab
INTYTGEPTYAADFKR

SEQ ID NO: 133 - protein, 14 aa, Artificial Sequence
  HCDR3 of Dilpacimab
YPHYYGSSHWYFDV

SEQ ID NO: 134 - protein, 11 aa, Artificial Sequence
  LCDR1 of Dilpacimab
SASQDISNYLN

SEQ ID NO: 135 - protein, 7 aa, Artificial Sequence
  LCDR2 of Dilpacimab
FTSSLHS

SEQ ID NO: 136 - protein, 8 aa, Artificial Sequence
  LCDR3 of Dilpacimab
QQYSTVPW

SEQ ID NO: 137 - protein, 10 aa, Artificial Sequence
  HCDR1 of hPV-19
GYSFTNSGIN

SEQ ID NO: 138 - protein, 14 aa, Artificial Sequence
  HCDR2 of hPV-19
INTYTGEPTYADDF

SEQ ID NO: 139 - protein, 10 aa, Artificial Sequence
  HCDR3 of hPV-19
FGDGYYWFFD

SEQ ID NO: 140 - protein, 17 aa, Artificial Sequence
  LCDR1 of hPV-19
KSSQSLLNSRTRKNFLA

SEQ ID NO: 141 - protein, 7 aa, Artificial Sequence
  LCDR2 of hPV-19
WASTRES

SEQ ID NO: 142 - protein, 11 aa, Artificial Sequence
  LCDR3 of hPV-19
KQSYNLYTFGG

SEQ ID NO: 143 - protein, 5 aa, Artificial Sequence
  HCDR1 of AT-001
SYAIS

SEQ ID NO: 144 - protein, 17 aa, Artificial Sequence
  HCDR2 of AT-001
GFDPEDGETIYAQKFQG

SEQ ID NO: 145 - protein, 17 aa, Artificial Sequence
  HCDR3 of AT-001
GRSMVRGVIIPFNGMDV

SEQ ID NO: 146 - protein, 11 aa, Artificial Sequence
  LCDR1 of AT-001
RASQSISSYLN

SEQ ID NO: 147 - protein, 7 aa, Artificial Sequence
  LCDR2 of AT-001
AASSLQS

SEQ ID NO: 148 - protein, 9 aa, Artificial Sequence
  LCDR3 of AT-001
QQSYSTPLT

SEQ ID NO: 149 - protein, 1673 aa, Artificial Sequence
  amino sequence of rabbit C3
MAEPWPLALMLLLCGSPLYRAEPLYILVTPRVLRLGSPENIHVQAHSESRERLQGSFKVNLTVWDFPLRKTLLASSRVVLSATNDFMEQTPVTVPESLLFPRHEKPGQHYVIIRADWKPTSVSSFMEKIVLVAPHAGYIFIQTDKTIYTPDHMVQYRVFAVNHKMDPVNRAILLDIKNPDGVTVISHSRQVINGLFDSSFHLPELVSLGTWTIEASYQSAGKQKFKATFDVKEYVLPSFEVQLTPNKTFFTLNDEALGVDIQARYIFNKPVDGHALAIFGLKVDNIRTTIQGSLQRVEVSEGQGHVSLQKDTLLAAFQDPEGDFSGASIFVNVTVFSSGGEMVQAETSGVKITRKAFNIKFTKTPQYFKPGMPFHFRVFVSNPDGSPAARVLVRCQNHKVYTSDNGIAALAINTDAASSELTVLVETESPHPEQQVSARMTAWPYSTQENSGNFLHVEVNTMGTDVGNSLQLSLNTRHANPATKDEITHFTIMVLSKGRVVSARQQLKSSGSVYTSAIIDVTPEMLPSFRIVAFYLLPRGMSQNPELVADSIWIDVNDRCMGTLKVGLKRDGVIQPLEPQSQVELKVTGDAEARVWLLAVDKAVYALNSKHKLTQKKVWDVVEEHDIGCTAGSGKNNFAVFKDAGLDLKISTGMDTLASSDWRCPQSPPPSRRRRSLRRLEAKRDAVNKFKTELERKCCEAGLKENPAGLACEERTRHVLHGPSCMAAFLDCCQLSETLTREAREERLLLGTTDDDDEFLDDIFLDDLPVRTLFPESWLWRSVTLPESASGTSHLLTLVSMPDSITTWEFVAVSLKAGRGLCVSDPFELTVMKSFFVDLKLPSSVVRNEQIQIQAVLYNFRSRQVKVRVEFPYKEPLCSASKPGAPSRQVVTVPPTSSKIVPFVLLPLELGEVEVEVKAVGPEARDHVKKTLLVRAGGQVQRLSHSFLLNPQGRTQTELVPRRELLNKVPDTEAEVFVSVQGDILGETIVGSLTPKETRKLLTVPTGCPEQTLSKLAPVIILTKYLDSTGQWSKVGVEHREQVLKNLVIGHTQMLRYRSADGIYRLTQNSPGSTWFTSYMFRIFALAYPIMTDKLPRLSELCAMAKWVITQRQAEDGHFLENGPVVMKSMQGGYKGSEADISLTALVLIALHSGQELCSPTMQNLDASIKRASNFLETKLPTIQTTFAIAIVSYALALANSPKANDRLDSFANYSHCGDCGEGAADKTYWPVGEPDEDSLYTIEATAYALMQKLQLGRFNETHAIANWLLEKRELGGGFKSTQTTVVAIEALTSFRKNVPFEGEQNLDVQISVPKRAVHVNWLINHNNAYQQRSAKFFSQDDLVITASGHGTGTISILTTYYKSPESWESPCTRYHLNVTLHSTPEANKKGEETFRLRMETRYLGAQDATMTIMEVSLLTGFYPNQEDLKQLTNNVEPYAFQYETKTSSSDSSVVLYLEKLSHQENTVLGFRIHQMLQADFLQAAMVTVYDYYEPSHRCSAFYNLPTERSSLRKICHKDVCRCAEGQCTALRTDSSRLSKEELQEAACEAGVDFVYKIKLEGVEASATTPYVYYNMRLQAVIKSGTDPVIPNTLKKFVSHATCHDSLDLQEQESYLVMGQTSDLWKVKSDYTYVLGKDTFLMLWPADGDVRRRKLLGELEEFSEYLTTHGCQS

SEQ ID NO: 150 - protein, 1639 aa, Artificial Sequence
  amino sequence of rat C3(25-1663)
SPMYSIITPNVLRLESEETFILEAHDAQGDVPVTVTVQDFLKKQVLTSEKTVLTGATGHLNRVFIKIPASKEFNADKGHKYVTVVANFGATVVEKAVLVSFQSGYLFIQTDKTIYTPGSTVFYRIFTVDNNLLPVGKTVVIVIETPDGVPIKRDILSSHNQYGILPLSWNIPELVNMGQWKIRAFYEHAPKQTFSAEFEVKEYVLPSFEVLVEPTEKFYYIHGPKGLEVSITARFLYGKNVDGTAFVIFGVQDEDKKISLALSLTRVLIEDGSGEAVLSRKVLMDGVRPSSPEALVGKSLYVSVTVILHSGSDMVEAERSGIPIVTSPYQIHFTKTPKFFKPAMPFDLMVFVTNPDGSPARRVPVVTQGSDAQALTQDDGVAKLSVNTPNNRQPLTITVSTKKEGIPDARQATRTMQAQPYSTMHNSNNYLHLSVSRVELKPGDNLNVNFHLRTDAGQEAKIRYYTYLVMNKGKLLKAGRQVREPGQDLVVLSLPITPEFIPSFRLVAYYTLIGANGQREVVADSVWVDVKDSCVGTLVVKGDPRDNRQPAPGHQTTLRIEGNQGARVGLVAVDKGVFVLNKKNKLTQSKIWDVVEKADIGCTPGSGKNYAGVFMDAGLTFKTNQGLQTDQREDPECAKPAARRRRSVQLMERRMDKAGQYTDKGLRKCCEDGMRDIPMPYSCQRRARLITQGESCLKAFMDCCNYITKLREQHRRDHVLGLARSDVDEDIIPEEDIISRSHFPESWLWTIEELKEPEKNGISTKVMNIFLKDSITTWEILAVSLSDKKGICVADPYEITVMQDFFIDLRLPYSVVRNEQVEIRAVLFNYREQEKLKVRVELLHNPAFCSMATAKKRYYQTIEIPPKSSVAVPYVIVPLKIGLQEVEVKAAVFNHFISDGVKKILKVVPEGMRVNKTVAVRTLDPEHLNQGGVQREDVNAADLSDQVPDTDSETRILLQGTPVAQMAEDAVDGERLKHLIVTPSGCGEQNMIGMTPTVIAVHYLDQTEQWEKFGLEKRQEALELIKKGYTQQLAFKQPISAYAAFNNRPPSTWLTAMWSRSFSLAANLIAIDSQVLCGAVKWLILEKQKPDGVFQEDGPVIHQEMIGGFRNTKEADVSLTAFVLIALQEARDICEGQVNSLPGSINKAGEYLEASYLNLQRPYTVAIAGYALALMNKLEEPYLTKFLNTAKDRNRWEEPGQQLYNVEATSYALLALLLLKDFDSVPPVVRWLNDERYYGGGYGSTQATFMVFQALAQYRADVPDHKDLNMDVSLHLPSRSSPTVFRLLWESGSLLRSEETKQNEGFSLTAKGKGQGTLSVVTVYHAKVKGKTTCKKFDLRVTIKPAPETAKKPQDAKSSMILDICTRYLGDVDATMSILDISMMTGFIPDTNDLELLSSGVDRYISKYEMDKAFSNKNTLIIYLEKISHSEEDCLSFKVHQFFNVGLIQPGSVKVYSYYNLEESCTRFYHPEKDDGMLSKLCHNEMCRCAEENCFMHQSQDQVSLNERLDKACEPGVDYVYKTKLTTIELSDDFDEYIMTIEQVIKSGSDEVQAGQERRFISHVKCRNALKLQKGKQYLMWGLSSDLWGEKPNTSYIIGKDTWVEHWPEAEERQDQKNQKQCEDLGAFTETMVVFGCPN

SEQ ID NO: 151 - protein, 321 aa, Artificial Sequence
  CRIg (VSIG4) isoform 2
MGILLGLLLLGHLTVDTYGRPILEVPESVTGPWKGDVNLPCTYDPLQGYTQVLVKWLVQRGSDPVTIFLRDSSGDHIQQAKYQGRLHVSHKVPGDVSLQLSTLEMDDRSHYTCEVTWQTPDGNQVVRDKITELRVQKLSVSKPTVTTGSGYGFTVPQGMRISLQCQARGSPPISYIWYKQQTNNQEPIKVATLSTLLFKPAVIADSGSYFCTAKGQVGSEQHSDIVKFVVKDSSKLLKTKTEAPTTMTYPLKATSTVKQSWDWTTDMDGYLGETSAGPGKSLPVFAIILIISLCCMVVFTMAYIMLCRKTSQQEHVYEAAR